European Patent Application EP 4 641 574 A1, published October 29, 2025. Title: METHOD FOR ESTIMATING ORGANISM OR HOST, METHOD FOR ACQUIRING MODEL FOR ESTIMATING ORGANISM OR HOST, AND COMPUTER DEVICE FOR PERFORMING SAME. Applicant: Seegene, Inc. Application EP 23 895 080.2, filed November 24, 2023. The sequence listing filed with the application follows.

SEQUENCE LISTING (17 sequences)

SEQ ID NO: 1 - DNA, 12 bp, synthetic construct
  source 1..12: mol_type = other DNA
attgacgattta

SEQ ID NO: 2 - DNA, 20 bp, synthetic construct
  source 1..20: mol_type = other DNA
acttcgagcgtatctgctag

SEQ ID NO: 3 - DNA, 141 bp, synthetic construct
  source 1..141: mol_type = other DNA
acgcgctcacagtcagcacagtttcgcagcctaacgcatcatgcatacatggcagtcacacacagcgccccatcatatagcatcaatgcatcagactgcagcatttcgcaagctcgctctactctacgttcaagctcggca

SEQ ID NO: 4 - DNA, 34 bp, synthetic construct
  source 1..34: mol_type = other DNA
acgcgctcacagtcagcacagtttcgcagcctaa

SEQ ID NO: 5 - DNA, 34 bp, synthetic construct
  source 1..34: mol_type = other DNA
atcatgcatacatggcagtcacacacagcgcccc

SEQ ID NO: 6 - DNA, 34 bp, synthetic construct
  source 1..34: mol_type = other DNA
gcaagctcgctctactctacgttcaagctcggca

SEQ ID NO: 7 - DNA, 19 bp, synthetic construct
  source 1..19: mol_type = other DNA
atgcacatcaccattcaca

SEQ ID NO: 8 - DNA, 18 bp, synthetic construct
  source 1..18: mol_type = other DNA
atcagtcacgcagtcagt

SEQ ID NO: 9 - DNA, 18 bp, synthetic construct
  source 1..18: mol_type = other DNA
gtcagtcagtcattcatc

SEQ ID NO: 10 - DNA, 19 bp, synthetic construct
  source 1..19: mol_type = other DNA
acgtatgcatatcatactt

SEQ ID NO: 11 - DNA, 18 bp, synthetic construct
  source 1..18: mol_type = other DNA
tcagcgtcgctcagatcg

SEQ ID NO: 12 - DNA, 40 bp, synthetic construct
  source 1..40: mol_type = other DNA
agcattgtgggtagtaaggtataaaagctcaaaatctaca

SEQ ID NO: 13 - DNA, 40 bp, synthetic construct
  source 1..40: mol_type = other DNA
agcgttattgttgagaaatggattgagcacaaaaaaattt

SEQ ID NO: 14 - DNA, 40 bp, synthetic construct
  source 1..40: mol_type = other DNA
agctgtttttttttttgttgtgggtaaagcctataaatcc

SEQ ID NO: 15 - DNA, 30 bp, synthetic construct
  source 1..30: mol_type = other DNA
attttgtgagacacgcgagatattttttta

SEQ ID NO: 16 - DNA, 30 bp, synthetic construct
  source 1..30: mol_type = other DNA
attttgtgngncncgcgagatattttttta

SEQ ID NO: 17 - DNA, 51 bp, synthetic construct
  source 1..51: mol_type = other DNA
atgtgcgcacacacacatatctcacacaccccacatattttctcacacaca